European Patent Specification EP 3 583 218 B1, published April 16, 2025. Title: FUSION PROTEIN AND LIGAND-PAYLOAD BASED DRUG DELIVERY FOR CELL THERAPY. Applicant: Purdue Research Foundation. The sequence listing filed with the application follows.

SEQUENCE LISTING (21 sequences)

SEQ ID NO: 1 - protein, 367 aa, artificial
  Amino acid sequence for mouse FKBP-FRa with linker peptide
MAHLMTVQLLLLVMWMAECAQSRAGVQVETISPGDGRTFPKRGQTCVVHYTGMLEDGKKFDSSRDRNKPFKFTLGKQEVIRGWEEGVAQMSVGQRAKLIISSDYAYGATGHPGIIPPHATLVFDVELLKLESGGGSTRARTELLNVCMDAKHHKEKPGPEDNLHDQCSPWKTNSCCSTNTSQEAHKDISYLYRFNWNHCGTMTSECKRHFIQDTCLYECSPNLGPWIQQVDQSWRKERILDVPLCKEDCQQWWEDCQSSFTCKSNWHKGWNWSSGHNECPVGASCHPFTFYFPTSAALCEEIWSHSYKLSNYSRGSGRCIQMWFDPAQGNPNEEVARFYAEAMSGAGFHGTWPLLCSLSLVLLWVIS

SEQ ID NO: 2 - protein, 369 aa, artificial
  Amino acid sequence for human FKBP-FRa with linker peptide
MAQRMTTQLLLLLVWVAVVGEAQTGVQVETISPGDGRTFPKRGQTCVVHYTGMLEDGKKFDSSRDRNKPFKFMLGKQEVIRGWEEGVAQMSVGQRAKLTISPDYAYGATGHPGIIPPHATLVFDVELLKLESGGGSRIAWARTELLNVCMNAKHHKEKPGPEDKLHEQCRPWRKNACCSTNTSQEAHKDVSYLYRFNWNHCGEMAPACKRHFIQDTCLYECSPNLGPWIQQVDQSWRKERVLNVPLCKEDCEQWWEDCRTSYTCKSNWHKGWNWTSGFNKCAVGAACQPFHFYFPTPTVLCNEIWTHSYKVSNYSRGSGRCIQMWFDPAQGNPNEEVARFYAAAMSGAGPWAAWPFLLSLALMLLWLLS

SEQ ID NO: 3 - protein, 485 aa, artificial
  Amino acid sequence for mouse antiCD19 CAR T construct
MGVPTQLLGLLLLWITDAICEQKLISEEDLDIQMTQSPASLSTSLGETVTIQCQASEDIYSGLAWYQQKPGKSPQLLIYGASDLQDGVPSRFSGSGSGTQYSLKITSMQTEDEGVYFCQQGLTYPRTFGGGTKLELKGGGGSGGGGSGGGGSEVQLQQSGAELVRPGTSVKLSCKVSGDTITFYYMHFVKQRPGQGLEWIGRIDPEDESTKYSEKFKNKATLTADTSSNTAYLKLSSLTSEDTATYFCIYGGYYFDYWGQGVMVTVSSIEFMYPPPYLDNERSNGTIIHIKEKHLCHTQSSPKLFWALVVVAGVLFCYGLLVTVALCVIWTNSRRNRGGQSDYMNMTPRRPGLTRKPYQPYAPARDFAAYRPRAKFSRSAETAANLQDPNQLYNELNLGRREEYDVLEKKRARDPEMGGKQQRRRNPQEGVYNALQKDKMAEAYSEIGTKGERRRGKGHDGLYQGLSTATKDTYDALHMQTLAPR

SEQ ID NO: 4 - protein, 496 aa, artificial
  Amino acid sequence for human antiCD19 CAR T construct
MALPVTALLLPLALLLHAARPEQKLISEEDLDIQMTQTTSSLSASLGDRVTISCRASQDISKYLNWYQQKPDGTVKLLIYHTSRLHSGVPSRFSGSGSGTDYSLTISNLEQEDIATYFCQQGNTLPYTFGGGTKLEITGGGGSGGGGSGGGGSEVKLQESGPGLVAPSQSLSVTCTVSGVSLPDYGVSWIRQPPRKGLEWLGVIWGSETTYYNSALKSRLTIIKDNSKSQVFLKMNSLQTDDTAIYYCAKHYYYGGSYAMDYWGQGTSVTVSSAAAIEVMYPPPYLDNEKSNGTIIHVKGKHLCPSPLFPGPSKPFWVLVVVGGVLACYSLLVTVAFIIFWVRSKRSRLLHSDYMNMTPRRPGPTRKHYQPYAPPRDFAAYRSRVKFSRSADAPAYQQGQNQLYNELNLGRREEYDVLDKRRGRDPEMGGKPQRRKNPQEGLYNELQKDKMAEAYSEIGMKGERRRGKGHDGLYQGLSTATKDTYDALHMQALPPR

SEQ ID NO: 5 - DNA, 12182 bp, artificial
  Vector sequence for pWPI for human T cell transduction
ttggaagggctaattcactcccaaagaagacaagatatccttgatctgtggatctaccacacacaaggctacttccctgattagcagaactacacaccagggccaggggtcagatatccactgacctttggatggtgctacaagctagtaccagttgagccagataaggtagaagaggccaataaaggagagaacaccagcttgttacaccctgtgagcctgcatgggatggatgacccggagagagaagtgttagagtggaggtttgacagccgcctagcatttcatcacgtggcccgagagctgcatccggagtacttcaagaactgctgatatcgagcttgctacaagggactttccgctggggactttccagggaggcgtggcctgggcgggactggggagtggcgagccctcagatcctgcatataagcagctgctttttgcctgtactgggtctctctggttagaccagatctgagcctgggagctctctggctaactagggaacccactgcttaagcctcaataaagcttgccttgagtgcttcaagtagtgtgtgcccgtctgttgtgtgactctggtaactagagatccctcagacccttttagtcagtgtggaaaatctctagcagtggcgcccgaacagggacttgaaagcgaaagggaaaccagaggagctctctcgacgcaggactcggcttgctgaagcgcgcacggcaagaggcgaggggcggcgactggtgagtacgccaaaaattttgactagcggaggctagaaggagagagatgggtgcgagagcgtcagtattaagcgggggagaattagatcgcgatgggaaaaaattcggttaaggccagggggaaagaaaaaatataaattaaaacatatagtatgggcaagcagggagctagaacgattcgcagttaatcctggcctgttagaaacatcagaaggctgtagacaaatactgggacagctacaaccatcccttcagacaggatcagaagaacttagatcattatataatacagtagcaaccctctattgtgtgcatcaaaggatagagataaaagacaccaaggaagctttagacaagatagaggaagagcaaaacaaaagtaagaccaccgcacagcaagcggccgctgatcttcagacctggaggaggagatatgagggacaattggagaagtgaattatataaatataaagtagtaaaaattgaaccattaggagtagcacccaccaaggcaaagagaagagtggtgcagagagaaaaaagagcagtgggaataggagctttgttccttgggttcttgggagcagcaggaagcactatgggcgcagcgtcaatgacgctgacggtacaggccagacaattattgtctggtatagtgcagcagcagaacaatttgctgagggctattgaggcgcaacagcatctgttgcaactcacagtctggggcatcaagcagctccaggcaagaatcctggctgtggaaagatacctaaaggatcaacagctcctggggatttggggttgctctggaaaactcatttgcaccactgctgtgccttggaatgctagttggagtaataaatctctggaacagatttggaatcacacgacctggatggagtgggacagagaaattaacaattacacaagcttaatacactccttaattgaagaatcgcaaaaccagcaagaaaagaatgaacaagaattattggaattagataaatgggcaagtttgtggaattggtttaacataacaaattggctgtggtatataaaattattcataatgatagtaggaggcttggtaggtttaagaatagtttttgctgtactttctatagtgaatagagttaggcagggatattcaccattatcgtttcagacccacctcccaaccccgaggggacccgacaggcccgaaggaatagaagaagaaggtggagagagagacagagacagatccattcgattagtgaacggatctcgacggtatcgatgtcgacgataagctttgcaaagatggataaagttttaaacagagaggaatctttgcagctaatggaccttctaggtcttgaaaggagtgggaattggctccggtgcccgtcagtgggcagagcgcacatcgcccacagtccccgagaagttggggggaggggtcggcaattgaaccggtgcctagagaaggtggcgcggggtaaactgggaaagtgatgtcgtgtactggctccgcctttttcccgagggtgggggagaaccgtatataagtgcagtagtcgccgtgaacgttctttttcgcaacgggtttgccgccagaacacaggtaagtgccgtgtgtggttcccgcgggcctggcctctttacgggttatggcccttgcgtgccttgaattacttccactggctgcagtacgtgattcttgatcccgagcttcgggttggaagtgggtgggagagttcgaggccttgcgcttaaggagccccttcgcctcgtgcttgagttgaggcctggcctgggcgctggggccgccgcgtgcgaatctggtggcaccttcgcgcctgtctcgctgctttcgataagtctctagccatttaaaatttttgatgacctgctgcgacgctttttttctggcaagatagtcttgtaaatgcgggccaagatctgcacactggtatttcggtttttggggccgcgggcggcgacggggcccgtgcgtcccagcgcacatgttcggcgaggcggggcctgcgagcgcggccaccgagaatcggacgggggtagtctcaagctggccggcctgctctggtgcctggcctcgcgccgccgtgtatcgccccgccctgggcggcaaggctggcccggtcggcaccagttgcgtgagcggaaagatggccgcttcccggccctgctgcagggagctcaaaatggaggacgcggcgctcgggagagcgggcgggtgagtcacccacacaaaggaaaagggcctttccgtcctcagccgtcgcttcatgtgactccacggagtaccgggcgccgtccaggcacctcgattagttctcgagcttttggagtacgtcgtctttaggttggggggaggggttttatgcgatggagtttccccacactgagtgggtggagactgaagttaggccagcttggcacttgatgtaattctccttggaatttgccctttttgagtttggatcttggttcattctcaagcctcagacagtggttcaaagtttttttcttccatttcaggtgtcgtgaggaatttcgacatttaaatttaattaatctcgacggtatcggttaacttttaaaagaaaaggggggattggggggtacagtgcaggggaaagaatagtagacataatagcaacagacatacaaactaaagaattacaaaaacaaattacaaaaattcaaaattttatcgatcacgagactagcctcgaggtttatggctcacctgatgactgtgcagttgttgctcctggtgatgtggatggccgaatgtgctcagtccagagctggagtgcaggtggagaccatctctcctggagacgggcgcaccttcccaaagcgcggccagacctgcgtggtgcactacacggggatgcttgaagatggaaagaaatttgattcctctcgggacagaaacaagccttttaagtttacactaggcaagcaggaggtgatccgaggctgggaggaaggggtagcccagatgagtgtgggtcagagagccaaactgataatctcctcagactatgcctatggagccaccgggcacccaggcatcatcccaccacatgccactcttgtttttgatgtggagcttctaaaactggaaagcggcggcggcagcactcgggccaggactgaacttctcaatgtctgcatggatgccaaacaccacaaagaaaaaccgggccctgaggacaatttacacgaccagtgcagcccctggaagacgaattcctgctgttccacgaacacaagccaggaagcacataaggacatttcctacctgtaccggttcaactggaaccactgcggaactatgacatcggaatgcaaacggcactttatccaagacacctgcctctatgagtgttccccgaacttgggaccctggatccagcaggtggaccagagctggcgcaaagagcggatccttgatgttcccctgtgcaaagaggactgtcagcagtggtgggaggactgccagagctcttttacctgcaagagcaattggcacaagggatggaactggtcctcggggcataacgagtgtcctgtgggagcctcctgccatcccttcaccttctacttccccacatctgctgctctgtgtgaggaaatctggagtcactcctacaagctcagcaactacagtcgagggagcggccgctgcattcagatgtggttcgacccagcccagggcaaccccaacgaggaagtggcgaggttctatgccgaggccatgagtggagctgggtttcatgggacctggccactcttgtgcagcctgtccttagtgctgctctgggtgatcagctgaaaactacgggctgcaggaattccgcccccccccccctaacgttactggccgaagccgcttggaataaggccggtgtgcgtttgtctatatgttattttccaccatattgccgtcttttggcaatgtgagggcccggaaacctggccctgtcttcttgacgagcattcctaggggtctttcccctctcgccaaaggaatgcaaggtctgttgaatgtcgtgaaggaagcagttcctctggaagcttcttgaagacaaacaacgtctgtagcgaccctttgcaggcagcggaaccccccacctggcgacaggtgcctctgcggccaaaagccacgtgtataagatacacctgcaaaggcggcacaaccccagtgccacgttgtgagttggatagttgtggaaagagtcaaatggctctcctcaagcgtattcaacaaggggctgaaggatgcccagaaggtaccccattgtatgggatctgatctggggcctcggtgcacatgctttacatgtgtttagtcgaggttaaaaaacgtctaggccccccgaaccacggggacgtggttttcctttgaaaaacacgatgataataccatggtgagcaagggcgaggagctgttcaccggggtggtgcccatcctggtcgagctggacggcgacgtaaacggccacaagttcagcgtgtccggcgagggcgagggcgatgccacctacggcaagctgaccctgaagttcatctgcaccaccggcaagctgcccgtgccctggcccaccctcgtgaccaccctgacctacggcgtgcagtgcttcagccgctaccccgaccacatgaagcagcacgacttcttcaagtccgccatgcccgaaggctacgtccaggagcgcaccatcttcttcaaggacgacggcaactacaagacccgcgccgaggtgaagttcgagggcgacaccctggtgaaccgcatcgagctgaagggcatcgacttcaaggaggacggcaacatcctggggcacaagctggagtacaactacaacagccacaacgtctatatcatggccgacaagcagaagaacggcatcaaggtgaacttcaagatccgccacaacatcgaggacggcagcgtgcagctcgccgaccactaccagcagaacacccccatcggcgacggccccgtgctgctgcccgacaaccactacctgagcacccagtccgccctgagcaaagaccccaacgagaagcgcgatcacatggtcctgctggagttcgtgaccgccgccgggatcactctcggcatggacgagctgtacaagtccggactcagatctcgactagctagtagctagctagctagtcgagctcaagcttcgaattcgatatcaagcttatcgcgataccgtcgacctcgagggaattccgataatcaacctctggattacaaaatttgtgaaagattgactggtattcttaactatgttgctccttttacgctatgtggatacgctgctttaatgcctttgtatcatgctattgcttcccgtatggctttcattttctcctccttgtataaatcctggttgctgtctctttatgaggagttgtggcccgttgtcaggcaacgtggcgtggtgtgcactgtgtttgctgacgcaacccccactggttggggcattgccaccacctgtcagctcctttccgggactttcgctttccccctccctattgccacggcggaactcatcgccgcctgccttgcccgctgctggacaggggctcggctgttgggcactgacaattccgtggtgttgtcggggaagctgacgtcctttccatggctgctcgcctgtgttgccacctggattctgcgcgggacgtccttctgctacgtcccttcggccctcaatccagcggaccttccttcccgcggcctgctgccggctctgcggcctcttccgcgtcttcgccttcgccctcagacgagtcggatctccctttgggccgcctccccgcatcgggaattcgagctcggtacctttaagaccaatgacttacaaggcagctgtagatcttagccactttttaaaagaaaaggggggactggaagggctaattcactcccaacgaagacaagatgggatcaattcaccatgggaataacttcgtatagcatacattatacgaagttatgctgctttttgcttgtactgggtctctctggttagaccagatctgagcctgggagctctctggctaactagggaacccactgcttaagcctcaataaagcttgccttgagtgcttcaagtagtgtgtgcccgtctgttgtgtgactctggtaactagagatccctcagacccttttagtcagtgtggaaaatctctagcagcatctagaattaattccgtgtattctatagtgtcacctaaatcgtatgtgtatgatacataaggttatgtattaattgtagccgcgttctaacgacaatatgtacaagcctaattgtgtagcatctggcttactgaagcagaccctatcatctctctcgtaaactgccgtcagagtcggtttggttggacgaaccttctgagtttctggtaacgccgtcccgcacccggaaatggtcagcgaaccaatcagcagggtcatcgctagccagatcctctacgccggacgcatcgtggccggcatcaccggcgccacaggtgcggttgctggcgcctatatcgccgacatcaccgatggggaagatcgggctcgccacttcgggctcatgagcgcttgtttcggcgtgggtatggtggcaggccccgtggccgggggactgttgggcgccatctccttgcatgcaccattccttgcggcggcggtgctcaacggcctcaacctactactgggctgcttcctaatgcaggagtcgcataagggagagcgtcgaatggtgcactctcagtacaatctgctctgatgccgcatagttaagccagccccgacacccgccaacacccgctgacgcgccctgacgggcttgtctgctcccggcatccgcttacagacaagctgtgaccgtctccgggagctgcatgtgtcagaggttttcaccgtcatcaccgaaacgcgcgagacgaaagggcctcgtgatacgcctatttttataggttaatgtcatgataataatggtttcttagacgtcaggtggcacttttcggggaaatgtgcgcggaacccctatttgtttatttttctaaatacattcaaatatgtatccgctcatgagacaataaccctgataaatgcttcaataatattgaaaaaggaagagtatgagtattcaacatttccgtgtcgcccttattcccttttttgcggcattttgccttcctgtttttgctcacccagaaacgctggtgaaagtaaaagatgctgaagatcagttgggtgcacgagtgggttacatcgaactggatctcaacagcggtaagatccttgagagttttcgccccgaagaacgttttccaatgatgagcacttttaaagttctgctatgtggcgcggtattatcccgtattgacgccgggcaagagcaactcggtcgccgcatacactattctcagaatgacttggttgagtactcaccagtcacagaaaagcatcttacggatggcatgacagtaagagaattatgcagtgctgccataaccatgagtgataacactgcggccaacttacttctgacaacgatcggaggaccgaaggagctaaccgcttttttgcacaacatgggggatcatgtaactcgccttgatcgttgggaaccggagctgaatgaagccataccaaacgacgagcgtgacaccacgatgcctgtagcaatggcaacaacgttgcgcaaactattaactggcgaactacttactctagcttcccggcaacaattaatagactggatggaggcggataaagttgcaggaccacttctgcgctcggcccttccggctggctggtttattgctgataaatctggagccggtgagcgtgggtctcgcggtatcattgcagcactggggccagatggtaagccctcccgtatcgtagttatctacacgacggggagtcaggcaactatggatgaacgaaatagacagatcgctgagataggtgcctcactgattaagcattggtaactgtcagaccaagtttactcatatatactttagattgatttaaaacttcatttttaatttaaaaggatctaggtgaagatcctttttgataatctcatgaccaaaatcccttaacgtgagttttcgttccactgagcgtcagaccccgtagaaaagatcaaaggatcttcttgagatcctttttttctgcgcgtaatctgctgcttgcaaacaaaaaaaccaccgctaccagcggtggtttgtttgccggatcaagagctaccaactctttttccgaaggtaactggcttcagcagagcgcagataccaaatactgtccttctagtgtagccgtagttaggccaccacttcaagaactctgtagcaccgcctacatacctcgctctgctaatcctgttaccagtggctgctgccagtggcgataagtcgtgtcttaccgggttggactcaagacgatagttaccggataaggcgcagcggtcgggctgaacggggggttcgtgcacacagcccagcttggagcgaacgacctacaccgaactgagatacctacagcgtgagcattgagaaagcgccacgcttcccgaagggagaaaggcggacaggtatccggtaagcggcagggtcggaacaggagagcgcacgagggagcttccagggggaaacgcctggtatctttatagtcctgtcgggtttcgccacctctgacttgagcgtcgatttttgtgatgctcgtcaggggggcggagcctatggaaaaacgccagcaacgcggcctttttacggttcctggccttttgctggccttttgctcacatgttctttcctgcgttatcccctgattctgtggataaccgtattaccgcctttgagtgagctgataccgctcgccgcagccgaacgaccgagcgcagcgagtcagtgagcgaggaagcggaagagcgcccaatacgcaaaccgcctctccccgcgcgttggccgattcattaatgcagctgtggaatgtgtgtcagttagggtgtggaaagtccccaggctccccagcaggcagaagtatgcaaagcatgcatctcaattagtcagcaaccaggtgtggaaagtccccaggctccccagcaggcagaagtatgcaaagcatgcatctcaattagtcagcaaccatagtcccgcccctaactccgcccatcccgcccctaactccgcccagttccgcccattctccgccccatggctgactaattttttttatttatgcagaggccgaggccgcctcggcctctgagctattccagaagtagtgaggaggcttttttggaggcctaggcttttgcaaaaagcttggacacaagacaggcttgcgagatatgtttgagaataccactttatcccgcgtcagggagaggcagtgcgtaaaaagacgcggactcatgtgaaatactggtttttagtgcgccagatctctataatctcgcgcaacctattttcccctcgaacactttttaagccgtagataaacaggctgggacacttcacatgagcgaaaaatacatcgtcacctgggacatgttgcagatccatgcacgtaaactcgcaagccgactgatgccttctgaacaatggaaaggcattattgccgtaagccgtggcggtctgtaccgggtgcgttactggcgcgtgaactgggtattcgtcatgtcgataccgtttgtatttccagctacgatcacgacaaccagcgcgagcttaaagtgctgaaacgcgcagaaggcgatggcgaaggcttcatcgttattgatgacctggtggataccggtggtactgcggttgcgattcgtgaaatgtatccaaaagcgcactttgtcaccatcttcgcaaaaccggctggtcgtccgctggttgatgactatgttgttgatatcccgcaagatacctggattgaacagccgtgggatatgggcgtcgtattcgtcccgccaatctccggtcgctaatcttttcaacgcctggcactgccgggcgttgttctttttaacttcaggcgggttacaatagtttccagtaagtattctggaggctgcatccatgacacaggcaaacctgagcgaaaccctgttcaaaccccgctttaaacatcctgaaacctcgacgctagtccgccgctttaatcacggcgcacaaccgcctgtgcagtcggcccttgatggtaaaaccatccctcactggtatcgcatgattaaccgtctgatgtggatctggcgcggcattgacccacgcgaaatcctcgacgtccaggcacgtattgtgatgagcgatgccgaacgtaccgacgatgatttatacgatacggtgattggctaccgtggcggcaactggatttatgagtgggccccggatctttgtgaaggaaccttacttctgtggtgtgacataattggacaaactacctacagagatttaaagctctaaggtaaatataaaatttttaagtgtataatgtgttaaactactgattctaattgtttgtgtattttagattccaacctatggaactgatgaatgggagcagtggtggaatgcctttaatgaggaaaacctgttttgctcagaagaaatgccatctagtgatgatgaggctactgctgactctcaacattctactcctccaaaaaagaagagaaaggtagaagaccccaaggactttccttcagaattgctaagttttttgagtcatgctgtgtttagtaatagaactcttgcttgctttgctatttacaccacaaaggaaaaagctgcactgctatacaagaaaattatggaaaaatattctgtaacctttataagtaggcataacagttataatcataacatactgttttttcttactccacacaggcatagagtgtctgctattaataactatgctcaaaaattgtgtacctttagctttttaatttgtaaaggggttaataaggaatatttgatgtatagtgccttgactagagatcataatcagccataccacatttgtagaggttttacttgctttaaaaaacctcccacacctccccctgaacctgaaacataaaatgaatgcaattgttgttgttaacttgtttattgcagcttataatggttacaaataaagcaatagcatcacaaatttcacaaataaagcatttttttcactgcattctagttgtggtttgtccaaactcatcaatgtatcttatcatgtctggatcaactggataactcaagctaaccaaaatcatcccaaacttcccaccccataccctattaccactgccaattacctagtggtttcatttactctaaacctgtgattcctctgaattattttcattttaaagaaattgtatttgttaaatatgtactacaaacttagtag

SEQ ID NO: 6 - DNA, 6939 bp, artificial
  pMP71 gb NotIEcoRI mouse antiCD19 for mouse T cell transduction
tcaaggttaggaacagagagacaggagaatatgggccaaacaggatatctgtggtaagcagttcctgccccggctcagggccaagaacagttggaacagcagaatatgggccaaacaggatatctgtggtaagcagttcctgccccggctcagggccaagaacagatggtccccagatgcggtcccgccctcagcagtttctagagaaccatcagatgtttccagggtgccccaaggacctgaaatgaccctgtgccttatttgaactaaccaatcagttcgcttctcgcttctgttcgcgcgcttctgctccccgagctcaataaaagagcccacaacccctcactcggcgcgccagtcctccgattgactgcgtcgcccgggtacccgtattcccaataaagcctcttgctgtttgcatccgaatcgtggactcgctgatccttgggagggtctcctcagattgattgactgcccacctcgggggtctttcatttggaggttccaccgagatttggagacccctgcccagggaccaccgacccccccgccgggaggtaagctggccagcggtcgtttcgtgtctgtctctgtctttgggcgtgtttgtgccggcatctaatgtttgcgcctgcgtctgtactagttggctaactagatctgtatctggcggtcccgcggaagaactgacgagttcgtattcccggccgcagcccctgggagacgtcccagcggcctcgggggcccgttttgtggcccattctgtatcagttaacctacccgagtcggactttttggagctccgccactgtccgaggggtacgtggctttgttgggggacgagagacagagacacttcccgcccccgtctgaatttttgctttcggttttacgccgaaaccgcgccgcgcgtcttgtctgctgcagcatcgttctgtgttgtctctgtctgactgtgtttctgtatttgtctgaaaattagctcgacaaagttaagtaatagtccctctctccaagctcacttacaggcatgggggttcccacccagctgttggggttgctgctcctctggatcactgatgccatctgcgaacagaagctcatttctgaagaagatctggacatacagatgacccagagtcctgccagcttgtccacatccctcggagagaccgtgacaattcaatgccaggcctctgaggacatatattctggattggcttggtaccagcaaaagccaggtaaaagtcctcagttgttgatatacggcgcttctgatttgcaagacggggtgccctcacgatttagcgggtctggaagtggcactcagtacagtctgaagattacttcaatgcaaacagaagacgagggtgtgtatttttgccaacaggggctgacctacccaaggacattcgggggcggtacaaagcttgaacttaagggcggcggtgggtctggaggtggtggatctggcggagggggaagtgaggtacagctgcaacagtccggcgccgaactcgttcgccctggaacctcagtcaaattgtcatgcaaggtgagtggcgacacaataaccttttactatatgcacttcgttaaacagaggccaggtcaaggtctggaatggataggcagaattgatccagaagatgagtccaccaaatactcagaaaagttcaaaaacaaagccactcttactgccgacacctcaagcaacacagcatatcttaagctcagttcacttaccagcgaagacaccgccacctatttttgtatttatggtggctattactttgactactgggggcaaggtgttatggtaacagtttcttccattgaattcatgtatccacccccctatttggataatgaacgatctaatgggactataatacatatcaaggaaaagcatctgtgtcatacccaaagttcccctaagcttttctgggccctcgtcgttgtggcaggagtgcttttttgctatggattgttggttactgtggctctctgcgtcatttggacaaatagtaggaggaatcgggggggacaatctgattacatgaacatgacaccacggaggccaggccttaccagaaagccctaccaaccttatgcaccagcacgagacttcgccgcatacaggccaagggctaagttttcccgcagcgccgaaaccgcagccaacctccaagatcctaatcagctctataacgaattgaatcttggccgcagagaggagtacgacgtacttgagaaaaagagagctagggaccctgaaatgggtgggaagcaacagcgaagaaggaacccacaggaaggggtgtataatgcccttcaaaaggataaaatggcagaggcatacagtgaaatcggaaccaagggggagagacgcagagggaaaggccatgacggcctttatcagggtttgtcaactgctactaaagacacttatgatgccttgcatatgcaaactctcgcacccagatgacgagcatcttaccgccatttattcccatatttgttctgtttttcttgatttgggtatacatttaaatgttaataaaacaaaatggtggggcaatcatttacattttatgggatatgtaattactagttcaggtgtattgccacaagacaaacatgttaagaaactttcccgttatttacgctctgttcctgttaatcaacctctggattacaaaatttgtgaaagattgactgatattcttaactatgttgctccttttacgctgtgtggatatgctgctttaatgcctctgtatcatgctattgcttcccgtacggctttcgttttctcctccttgtataaatcctggttgctgtctctttatgaggagttgtggcccgttgtccgtcaacgtggcgtggtgtgctctgtgtttgctgacgcaacccccactggctggggcattgccaccacctgtcaactcctttctgggactttcgctttccccctcccgatcgccacggcagaactcatcgccgcctgccttgcccgctgctggacaggggctaggttgctgggcactgataattccgtggtgttgtcggggaagctgacgtcctttccatggctgctcgcctgtgttgccaactggatcctgcgcgggacgtccttctgctacgtcccttcggctctcaatccagcggacctcccttcccgaggccttctgccggttctgcggcctctcccgcgtcttcgctttcggcctccgacgagtcggatctccctttgggccgcctccccgcctgtttcgcctcggcgtccggtccgtgttgcttggtcgtcacctgtgcagaattgcgaaccatggattccaccgtgaactttgtctcctggcatgcaaatcgtcaacttggcatgccaagaattaattcggatccaagcttaggcctgctcgctttcttgctgtcccatttctattaaaggttcctttgttccctaagtccaactactaaactgggggatattatgaagggccttgagcatctggattctgcctagcgctaagcttcctaacacgagccatagatagaataaaagattttatttagtctccagaaaaaggggggaatgaaagaccccacctgtaggtttggcaagctagcttaagtaagccattttgcaaggcatggaaaaatacataactgagaatagagaagttcagatcaaggttaggaacagagagacaggagaatatgggccaaacaggatatctgtggtaagcagttcctgccccggctcagggccaagaacagttggaacagcagaatatgggccaaacaggatatctgtggtaagcagttcctgccccggctcagggccaagaacagatggtccccagatgcggtcccgccctcagcagtttctagagaaccatcagatgtttccagggtgccccaaggacctgaaatgaccctgtgccttatttgaactaaccaatcagttcgcttctcgcttctgttcgcgcgcttctgctccccgagctcaataaaagagcccacaacccctcactcggcgcgccagtcctccgatagactgcgtcgcccggggtacccgtattcccaataaagcctcttgctgtttgcatccgaatcgtggactcgctgatccttgggagggtctcctcagattgattgactgcccacctcgggggtctttcattctcgagagctttggcgtaatcatggtcatagctgtttcctgtgtgaaattgttatccgctcacaattccacacaacatacgagccggaagcataaagtgtaaagcctggggtgcctaatgagtgagctaactcacattaattgcgttgcgctcactgcccgctttccagtcgggaaacctgtcgtgccagctgcattaatgaatcggccaacgcgcggggagaggcggtttgcgtattgggcgctcttccgcttcctcgctcactgactcgctgcgctcggtcgttcggctgcggcgagcggtatcagctcactcaaaggcggtaatacggttatccacagaatcaggggataacgcaggaaagaacatgtgagcaaaaggccagcaaaaggccaggaaccgtaaaaaggccgcgttgctggcgtttttccataggctccgcccccctgacgagcatcacaaaaatcgacgctcaagtcagaggtggcgaaacccgacaggactataaagataccaggcgtttccccctggaagctccctcgtgcgctctcctgttccgaccctgccgcttaccggatacctgtccgcctttctcccttcgggaagcgtggcgctttctcaatgctcacgctgtaggtatctcagttcggtgtaggtcgttcgctccaagctgggctgtgtgcacgaaccccccgttcagcccgaccgctgcgccttatccggtaactatcgtcttgagtccaacccggtaagacacgacttatcgccactggcagcagccactggtaacaggattagcagagcgaggtatgtaggcggtgctacagagttcttgaagtggtggcctaactacggctacactagaaggacagtatttggtatctgcgctctgctgaagccagttaccttcggaaaaagagttggtagctcttgatccggcaaacaaaccaccgctggtagcggtggtttttttgtttgcaagcagcagattacgcgcagaaaaaaaggatctcaagaagatcctttgatcttttctacggggtctgacgctcagtggaacgaaaactcacgttaagggattttggtcatgagattatcaaaaaggatcttcacctagatccttttaaattaaaaatgaagttttaaatcaatctaaagtatatatgagtaaacttggtctgacagttaccaatgcttaatcagtgaggcacctatctcagcgatctgtctatttcgttcatccatagttgcctgactccccgtcgtgtagataactacgatacgggagggcttaccatctggccccagtgctgcaatgataccgcgagacccacgctcaccggctccagatttatcagcaataaaccagccagccggaagggccgagcgcagaagtggtcctgcaactttatccgcctccatccagtctattaattgttgccgggaagctagagtaagtagttcgccagttaatagtttgcgcaacgttgttgccattgctgctggcatcgtggtgtcacgctcgtcgtttggtatggcttcattcagctccggttcccaacgatcaaggcgagttacatgatcccccatgttgtgcaaaaaagcggttagctccttcggtcctccgatcgttgtcagaagtaagttggccgcagtgttatcactcatggttatggcagcactgcataattctcttactgtcatgccatccgtaagatgcttttctgtgactggtgagtactcaaccaagtcattctgagaatagtgtatgcggcgaccgagttgctcttgcccggcgtcaatacgggataataccgcgccacatagcagaactttaaaagtgctcatcattggaaaacgttcttcggggcgaaaactctcaaggatcttaccgctgttgagatccagttcgatgtaacccactcgtgcacccaactgatcttcagcatcttttactttcaccagcgtttctgggtgagcaaaaacaggaaggcaaaatgccgcaaaaaagggaataagggcgacacggaaatgttgaatactcatactcttcctttttcaatattattgaagcatttatcagggttattgtctcatgagcggatacatatttgaatgtatttagaaaaataaacaaataggggttccgcgcacatttccccgaaaagtgccacctgacgtctaagaaaccattattatcatgacattaacctataaaaataggcgtatcacgaggccctttcgtcttcaagctgcctcgcgcgtttcggtgatgacggtgaaaacctctgacacatgcagctcccggagacggtcacagcttgtctgtaagcggatgccgggagcagacaagcccgtcagggcgcgtcagcgggtgttggcgggtgtcggggcgcagccatgacccagtcacgtagcgatagttactatgcggcatcagagcagattgtactgagagtgcaccatatgcggtgtgaaataccgcacagatgcgtaaggagaaaataccgcatcaggcgccattcgccattcaggctgcgcaactgttgggaagggcgatcggtgcgggcctcttcgctattacgccagctggcgaaagggggatgtgctgcaaggcgattaagttgggtaacgccagggttttcccagtcacgacgttgtaaaacgacggccagtgaattagtactctagcttaagtaagccattttgcaaggcatggaaaaatacataactgagaatagagaagttcaga

SEQ ID NO: 7 - DNA, 12188 bp, artificial
  pWPI-FRa 1-24 FKBP FRa
ttggaagggctaattcactcccaaagaagacaagatatccttgatctgtggatctaccacacacaaggctacttccctgattagcagaactacacaccagggccaggggtcagatatccactgacctttggatggtgctacaagctagtaccagttgagccagataaggtagaagaggccaataaaggagagaacaccagcttgttacaccctgtgagcctgcatgggatggatgacccggagagagaagtgttagagtggaggtttgacagccgcctagcatttcatcacgtggcccgagagctgcatccggagtacttcaagaactgctgatatcgagcttgctacaagggactttccgctggggactttccagggaggcgtggcctgggcgggactggggagtggcgagccctcagatcctgcatataagcagctgctttttgcctgtactgggtctctctggttagaccagatctgagcctgggagctctctggctaactagggaacccactgcttaagcctcaataaagcttgccttgagtgcttcaagtagtgtgtgcccgtctgttgtgtgactctggtaactagagatccctcagacccttttagtcagtgtggaaaatctctagcagtggcgcccgaacagggacttgaaagcgaaagggaaaccagaggagctctctcgacgcaggactcggcttgctgaagcgcgcacggcaagaggcgaggggcggcgactggtgagtacgccaaaaattttgactagcggaggctagaaggagagagatgggtgcgagagcgtcagtattaagcgggggagaattagatcgcgatgggaaaaaattcggttaaggccagggggaaagaaaaaatataaattaaaacatatagtatgggcaagcagggagctagaacgattcgcagttaatcctggcctgttagaaacatcagaaggctgtagacaaatactgggacagctacaaccatcccttcagacaggatcagaagaacttagatcattatataatacagtagcaaccctctattgtgtgcatcaaaggatagagataaaagacaccaaggaagctttagacaagatagaggaagagcaaaacaaaagtaagaccaccgcacagcaagcggccgctgatcttcagacctggaggaggagatatgagggacaattggagaagtgaattatataaatataaagtagtaaaaattgaaccattaggagtagcacccaccaaggcaaagagaagagtggtgcagagagaaaaaagagcagtgggaataggagctttgttccttgggttcttgggagcagcaggaagcactatgggcgcagcgtcaatgacgctgacggtacaggccagacaattattgtctggtatagtgcagcagcagaacaatttgctgagggctattgaggcgcaacagcatctgttgcaactcacagtctggggcatcaagcagctccaggcaagaatcctggctgtggaaagatacctaaaggatcaacagctcctggggatttggggttgctctggaaaactcatttgcaccactgctgtgccttggaatgctagttggagtaataaatctctggaacagatttggaatcacacgacctggatggagtgggacagagaaattaacaattacacaagcttaatacactccttaattgaagaatcgcaaaaccagcaagaaaagaatgaacaagaattattggaattagataaatgggcaagtttgtggaattggtttaacataacaaattggctgtggtatataaaattattcataatgatagtaggaggcttggtaggtttaagaatagtttttgctgtactttctatagtgaatagagttaggcagggatattcaccattatcgtttcagacccacctcccaaccccgaggggacccgacaggcccgaaggaatagaagaagaaggtggagagagagacagagacagatccattcgattagtgaacggatctcgacggtatcgatgtcgacgataagctttgcaaagatggataaagttttaaacagagaggaatctttgcagctaatggaccttctaggtcttgaaaggagtgggaattggctccggtgcccgtcagtgggcagagcgcacatcgcccacagtccccgagaagttggggggaggggtcggcaattgaaccggtgcctagagaaggtggcgcggggtaaactgggaaagtgatgtcgtgtactggctccgcctttttcccgagggtgggggagaaccgtatataagtgcagtagtcgccgtgaacgttctttttcgcaacgggtttgccgccagaacacaggtaagtgccgtgtgtggttcccgcgggcctggcctctttacgggttatggcccttgcgtgccttgaattacttccactggctgcagtacgtgattcttgatcccgagcttcgggttggaagtgggtgggagagttcgaggccttgcgcttaaggagccccttcgcctcgtgcttgagttgaggcctggcctgggcgctggggccgccgcgtgcgaatctggtggcaccttcgcgcctgtctcgctgctttcgataagtctctagccatttaaaatttttgatgacctgctgcgacgctttttttctggcaagatagtcttgtaaatgcgggccaagatctgcacactggtatttcggtttttggggccgcgggcggcgacggggcccgtgcgtcccagcgcacatgttcggcgaggcggggcctgcgagcgcggccaccgagaatcggacgggggtagtctcaagctggccggcctgctctggtgcctggcctcgcgccgccgtgtatcgccccgccctgggcggcaaggctggcccggtcggcaccagttgcgtgagcggaaagatggccgcttcccggccctgctgcagggagctcaaaatggaggacgcggcgctcgggagagcgggcgggtgagtcacccacacaaaggaaaagggcctttccgtcctcagccgtcgcttcatgtgactccacggagtaccgggcgccgtccaggcacctcgattagttctcgagcttttggagtacgtcgtctttaggttggggggaggggttttatgcgatggagtttccccacactgagtgggtggagactgaagttaggccagcttggcacttgatgtaattctccttggaatttgccctttttgagtttggatcttggttcattctcaagcctcagacagtggttcaaagtttttttcttccatttcaggtgtcgtgaggaatttcgacatttaaatttaattaatctcgacggtatcggttaacttttaaaagaaaaggggggattggggggtacagtgcaggggaaagaatagtagacataatagcaacagacatacaaactaaagaattacaaaaacaaattacaaaaattcaaaattttatcgatcacgagactagcctcgaggtttatggctcagcggatgacaacacagctgctgctccttctagtgtgggtggctgtagtaggggaggctcagacaggagtgcaggtggagactatctccccaggagacgggcgcaccttccccaagcgcggccagacctgcgtggtgcactacaccgggatgcttgaagatggaaagaaatttgattcctcccgggacagaaacaagccctttaagtttatgctaggcaagcaggaggtgatccgaggctgggaagaaggggttgcccagatgagtgtgggtcagagagccaaactgactatatctccagattatgcctatggtgccactgggcacccaggcatcatcccaccacatgccactctcgtcttcgatgtggagcttctaaaactggaatctggcggtggatccaggattgcatgggccaggactgagcttctcaatgtctgcatgaacgccaagcaccacaaggaaaagccaggccccgaggacaagttgcatgagcagtgtcgaccctggaggaagaatgcctgctgttctaccaacaccagccaggaagcccataaggatgtttcctacctatatagattcaactggaaccactgtggagagatggcacctgcctgcaaacggcatttcatccaggacacctgcctctacgagtgctcccccaacttggggccctggatccagcaggtggatcagagctggcgcaaagagcgggtactgaacgtgcccctgtgcaaagaggactgtgagcaatggtgggaagattgtcgcacctcctacacctgcaagagcaactggcacaagggctggaactggacttcagggtttaacaagtgcgcagtgggagctgcctgccaacctttccatttctacttccccacacccactgttctgtgcaatgaaatctggactcactcctacaaggtcagcaactacagccgagggagtggccgctgcatccagatgtggttcgacccagcccagggcaaccccaatgaggaggtggcgaggttctatgctgcagccatgagtggggctgggccctgggcagcctggcctttcctgcttagcctggccctaatgctgctgtggctgctcagctgaaaactacgggctgcaggaattccgcccccccccccctaacgttactggccgaagccgcttggaataaggccggtgtgcgtttgtctatatgttattttccaccatattgccgtcttttggcaatgtgagggcccggaaacctggccctgtcttcttgacgagcattcctaggggtctttcccctctcgccaaaggaatgcaaggtctgttgaatgtcgtgaaggaagcagttcctctggaagcttcttgaagacaaacaacgtctgtagcgaccctttgcaggcagcggaaccccccacctggcgacaggtgcctctgcggccaaaagccacgtgtataagatacacctgcaaaggcggcacaaccccagtgccacgttgtgagttggatagttgtggaaagagtcaaatggctctcctcaagcgtattcaacaaggggctgaaggatgcccagaaggtaccccattgtatgggatctgatctggggcctcggtgcacatgctttacatgtgtttagtcgaggttaaaaaacgtctaggccccccgaaccacggggacgtggttttcctttgaaaaacacgatgataataccatggtgagcaagggcgaggagctgttcaccggggtggtgcccatcctggtcgagctggacggcgacgtaaacggccacaagttcagcgtgtccggcgagggcgagggcgatgccacctacggcaagctgaccctgaagttcatctgcaccaccggcaagctgcccgtgccctggcccaccctcgtgaccaccctgacctacggcgtgcagtgcttcagccgctaccccgaccacatgaagcagcacgacttcttcaagtccgccatgcccgaaggctacgtccaggagcgcaccatcttcttcaaggacgacggcaactacaagacccgcgccgaggtgaagttcgagggcgacaccctggtgaaccgcatcgagctgaagggcatcgacttcaaggaggacggcaacatcctggggcacaagctggagtacaactacaacagccacaacgtctatatcatggccgacaagcagaagaacggcatcaaggtgaacttcaagatccgccacaacatcgaggacggcagcgtgcagctcgccgaccactaccagcagaacacccccatcggcgacggccccgtgctgctgcccgacaaccactacctgagcacccagtccgccctgagcaaagaccccaacgagaagcgcgatcacatggtcctgctggagttcgtgaccgccgccgggatcactctcggcatggacgagctgtacaagtccggactcagatctcgactagctagtagctagctagctagtcgagctcaagcttcgaattcgatatcaagcttatcgcgataccgtcgacctcgagggaattccgataatcaacctctggattacaaaatttgtgaaagattgactggtattcttaactatgttgctccttttacgctatgtggatacgctgctttaatgcctttgtatcatgctattgcttcccgtatggctttcattttctcctccttgtataaatcctggttgctgtctctttatgaggagttgtggcccgttgtcaggcaacgtggcgtggtgtgcactgtgtttgctgacgcaacccccactggttggggcattgccaccacctgtcagctcctttccgggactttcgctttccccctccctattgccacggcggaactcatcgccgcctgccttgcccgctgctggacaggggctcggctgttgggcactgacaattccgtggtgttgtcggggaagctgacgtcctttccatggctgctcgcctgtgttgccacctggattctgcgcgggacgtccttctgctacgtcccttcggccctcaatccagcggaccttccttcccgcggcctgctgccggctctgcggcctcttccgcgtcttcgccttcgccctcagacgagtcggatctccctttgggccgcctccccgcatcgggaattcgagctcggtacctttaagaccaatgacttacaaggcagctgtagatcttagccactttttaaaagaaaaggggggactggaagggctaattcactcccaacgaagacaagatgggatcaattcaccatgggaataacttcgtatagcatacattatacgaagttatgctgctttttgcttgtactgggtctctctggttagaccagatctgagcctgggagctctctggctaactagggaacccactgcttaagcctcaataaagcttgccttgagtgcttcaagtagtgtgtgcccgtctgttgtgtgactctggtaactagagatccctcagacccttttagtcagtgtggaaaatctctagcagcatctagaattaattccgtgtattctatagtgtcacctaaatcgtatgtgtatgatacataaggttatgtattaattgtagccgcgttctaacgacaatatgtacaagcctaattgtgtagcatctggcttactgaagcagaccctatcatctctctcgtaaactgccgtcagagtcggtttggttggacgaaccttctgagtttctggtaacgccgtcccgcacccggaaatggtcagcgaaccaatcagcagggtcatcgctagccagatcctctacgccggacgcatcgtggccggcatcaccggcgccacaggtgcggttgctggcgcctatatcgccgacatcaccgatggggaagatcgggctcgccacttcgggctcatgagcgcttgtttcggcgtgggtatggtggcaggccccgtggccgggggactgttgggcgccatctccttgcatgcaccattccttgcggcggcggtgctcaacggcctcaacctactactgggctgcttcctaatgcaggagtcgcataagggagagcgtcgaatggtgcactctcagtacaatctgctctgatgccgcatagttaagccagccccgacacccgccaacacccgctgacgcgccctgacgggcttgtctgctcccggcatccgcttacagacaagctgtgaccgtctccgggagctgcatgtgtcagaggttttcaccgtcatcaccgaaacgcgcgagacgaaagggcctcgtgatacgcctatttttataggttaatgtcatgataataatggtttcttagacgtcaggtggcacttttcggggaaatgtgcgcggaacccctatttgtttatttttctaaatacattcaaatatgtatccgctcatgagacaataaccctgataaatgcttcaataatattgaaaaaggaagagtatgagtattcaacatttccgtgtcgcccttattcccttttttgcggcattttgccttcctgtttttgctcacccagaaacgctggtgaaagtaaaagatgctgaagatcagttgggtgcacgagtgggttacatcgaactggatctcaacagcggtaagatccttgagagttttcgccccgaagaacgttttccaatgatgagcacttttaaagttctgctatgtggcgcggtattatcccgtattgacgccgggcaagagcaactcggtcgccgcatacactattctcagaatgacttggttgagtactcaccagtcacagaaaagcatcttacggatggcatgacagtaagagaattatgcagtgctgccataaccatgagtgataacactgcggccaacttacttctgacaacgatcggaggaccgaaggagctaaccgcttttttgcacaacatgggggatcatgtaactcgccttgatcgttgggaaccggagctgaatgaagccataccaaacgacgagcgtgacaccacgatgcctgtagcaatggcaacaacgttgcgcaaactattaactggcgaactacttactctagcttcccggcaacaattaatagactggatggaggcggataaagttgcaggaccacttctgcgctcggcccttccggctggctggtttattgctgataaatctggagccggtgagcgtgggtctcgcggtatcattgcagcactggggccagatggtaagccctcccgtatcgtagttatctacacgacggggagtcaggcaactatggatgaacgaaatagacagatcgctgagataggtgcctcactgattaagcattggtaactgtcagaccaagtttactcatatatactttagattgatttaaaacttcatttttaatttaaaaggatctaggtgaagatcctttttgataatctcatgaccaaaatcccttaacgtgagttttcgttccactgagcgtcagaccccgtagaaaagatcaaaggatcttcttgagatcctttttttctgcgcgtaatctgctgcttgcaaacaaaaaaaccaccgctaccagcggtggtttgtttgccggatcaagagctaccaactctttttccgaaggtaactggcttcagcagagcgcagataccaaatactgtccttctagtgtagccgtagttaggccaccacttcaagaactctgtagcaccgcctacatacctcgctctgctaatcctgttaccagtggctgctgccagtggcgataagtcgtgtcttaccgggttggactcaagacgatagttaccggataaggcgcagcggtcgggctgaacggggggttcgtgcacacagcccagcttggagcgaacgacctacaccgaactgagatacctacagcgtgagcattgagaaagcgccacgcttcccgaagggagaaaggcggacaggtatccggtaagcggcagggtcggaacaggagagcgcacgagggagcttccagggggaaacgcctggtatctttatagtcctgtcgggtttcgccacctctgacttgagcgtcgatttttgtgatgctcgtcaggggggcggagcctatggaaaaacgccagcaacgcggcctttttacggttcctggccttttgctggccttttgctcacatgttctttcctgcgttatcccctgattctgtggataaccgtattaccgcctttgagtgagctgataccgctcgccgcagccgaacgaccgagcgcagcgagtcagtgagcgaggaagcggaagagcgcccaatacgcaaaccgcctctccccgcgcgttggccgattcattaatgcagctgtggaatgtgtgtcagttagggtgtggaaagtccccaggctccccagcaggcagaagtatgcaaagcatgcatctcaattagtcagcaaccaggtgtggaaagtccccaggctccccagcaggcagaagtatgcaaagcatgcatctcaattagtcagcaaccatagtcccgcccctaactccgcccatcccgcccctaactccgcccagttccgcccattctccgccccatggctgactaattttttttatttatgcagaggccgaggccgcctcggcctctgagctattccagaagtagtgaggaggcttttttggaggcctaggcttttgcaaaaagcttggacacaagacaggcttgcgagatatgtttgagaataccactttatcccgcgtcagggagaggcagtgcgtaaaaagacgcggactcatgtgaaatactggtttttagtgcgccagatctctataatctcgcgcaacctattttcccctcgaacactttttaagccgtagataaacaggctgggacacttcacatgagcgaaaaatacatcgtcacctgggacatgttgcagatccatgcacgtaaactcgcaagccgactgatgccttctgaacaatggaaaggcattattgccgtaagccgtggcggtctgtaccgggtgcgttactggcgcgtgaactgggtattcgtcatgtcgataccgtttgtatttccagctacgatcacgacaaccagcgcgagcttaaagtgctgaaacgcgcagaaggcgatggcgaaggcttcatcgttattgatgacctggtggataccggtggtactgcggttgcgattcgtgaaatgtatccaaaagcgcactttgtcaccatcttcgcaaaaccggctggtcgtccgctggttgatgactatgttgttgatatcccgcaagatacctggattgaacagccgtgggatatgggcgtcgtattcgtcccgccaatctccggtcgctaatcttttcaacgcctggcactgccgggcgttgttctttttaacttcaggcgggttacaatagtttccagtaagtattctggaggctgcatccatgacacaggcaaacctgagcgaaaccctgttcaaaccccgctttaaacatcctgaaacctcgacgctagtccgccgctttaatcacggcgcacaaccgcctgtgcagtcggcccttgatggtaaaaccatccctcactggtatcgcatgattaaccgtctgatgtggatctggcgcggcattgacccacgcgaaatcctcgacgtccaggcacgtattgtgatgagcgatgccgaacgtaccgacgatgatttatacgatacggtgattggctaccgtggcggcaactggatttatgagtgggccccggatctttgtgaaggaaccttacttctgtggtgtgacataattggacaaactacctacagagatttaaagctctaaggtaaatataaaatttttaagtgtataatgtgttaaactactgattctaattgtttgtgtattttagattccaacctatggaactgatgaatgggagcagtggtggaatgcctttaatgaggaaaacctgttttgctcagaagaaatgccatctagtgatgatgaggctactgctgactctcaacattctactcctccaaaaaagaagagaaaggtagaagaccccaaggactttccttcagaattgctaagttttttgagtcatgctgtgtttagtaatagaactcttgcttgctttgctatttacaccacaaaggaaaaagctgcactgctatacaagaaaattatggaaaaatattctgtaacctttataagtaggcataacagttataatcataacatactgttttttcttactccacacaggcatagagtgtctgctattaataactatgctcaaaaattgtgtacctttagctttttaatttgtaaaggggttaataaggaatatttgatgtatagtgccttgactagagatcataatcagccataccacatttgtagaggttttacttgctttaaaaaacctcccacacctccccctgaacctgaaacataaaatgaatgcaattgttgttgttaacttgtttattgcagcttataatggttacaaataaagcaatagcatcacaaatttcacaaataaagcatttttttcactgcattctagttgtggtttgtccaaactcatcaatgtatcttatcatgtctggatcaactggataactcaagctaaccaaaatcatcccaaacttcccaccccataccctattaccactgccaattacctagtggtttcatttactctaaacctgtgattcctctgaattattttcattttaaagaaattgtatttgttaaatatgtactacaaacttagtag

SEQ ID NO: 8 - DNA, 12182 bp, artificial; identical to SEQ ID NO: 5
  pWPI mFKBP-mFRa SGGGS

SEQ ID NO: 9 - DNA, 10447 bp, artificial
  pHR EcorI hAnti cd19 1D3 myc hinge cd28 cd3zeta
cgataccgtcgaccaaggcagctgtagatcttagccactttttaaaagaaaaggggggactggaagggctaattcactcccaacgaagacaagatctgctttttgcttgtactgggtctctctggttagaccagatctgagcctgggagctctctggctaactagggaacccactgcttaagcctcaataaagcttgccttgagtgcttcaagtagtgtgtgcccgtctgttgtgtgactctggtaactagagatccctcagacccttttagtcagtgtggaaaatctctagcagcatctagaattaattccgtgtattctatagtgtcacctaaatcgtatgtgtatgatacataaggttatgtattaattgtagccgcgttctaacgacaatatgtacaagcctaattgtgtagcatctggcttactgaagcagaccctatcatctctctcgtaaactgccgtcagagtcggtttggttggacgaaccttctgagtttctggtaacgccgtcccgcacccggaaatggtcagcgaaccaatcagcagggtcatcgctagccagatcctctacgccggacgcatcgtggccggcatcaccggcgccacaggtgcggttgctggcgcctatatcgccgacatcaccgatggggaagatcgggctcgccacttcgggctcatgagcgcttgtttcggcgtgggtatggtggcaggccccgtggccgggggactgttgggcgccatctccttgcatgcaccattccttgcggcggcggtgctcaacggcctcaacctactactgggctgcttcctaatgcaggagtcgcataagggagagcgtcgaatggtgcactctcagtacaatctagctctgatgccgcatagttaagccagccccgacacccgccaacacccgctgacgcgccctgacgggcttgtctgctcccggcatccgcttacagacaagctgtgaccgtctccgggagctgcatgtgtcagaggttttcaccgtcatcaccgaaacgcgcgagacgaaagggcctcgtgatacgcctatttttataggttaatgtcatgataataatggtttcttagacgtcaggtggcacttttcggggaaatgtgcgcggaacccctatttgtttatttttctaaatacattcaaatatgtatccgctcatgagacaataaccctgataaatgcttcaataatattgaaaaaggaagagtatgagtattcaacatttccgtgtcgcccttattcccttttttgcggcattttgccttcctgtttttgctcacccagaaacgctggtgaaagtaaaagatgctgaagatcagttgggtgcacgagtgggttacatcgaactggatctcaacagcggtaagatccttgagagttttcgccccgaagaacgttttccaatgatgagcacttttaaagttctgctatgtggcgcggtattatcccgtattgacgccgggcaagagcaactcggtcgccgcatacactattctcagaatgacttggttgagtactcaccagtcacagaaaagcatcttacggatggcatgacagtaagagaattatgcagtgctgccataaccatgagtgataacactgcggccaacttacttctgacaacgatcggaggaccgaaggagctaaccgcttttttgcacaacatgggggatcatgtaactcgccttgatcgttgggaaccggagctgaatgaagccataccaaacgacgagcgtgacaccacgatgcctgtagcaatggcaacaacgttgcgcaaactattaactggcgaactacttactctagcttcccggcaacaattaatagactggatggaggcggataaagttgcaggaccacttctgcgctcggcccttccggctggctggtttattgctgataaatctggagccggtgagcgtgggtctcgcggtatcattgcagcactggggccagatggtaagccctcccgtatcgtagttatctacacgacggggagtcaggcaactatggatgaacgaaatagacagatcgctgagataggtgcctcactgattaagcattggtaactgtcagaccaagtttactcatatatactttagattgatttaaaacttcatttttaatttaaaaggatctaggtgaagatcctttttgataatctcatgaccaaaatcccttaacgtgagttttcgttccactgagcgtcagaccccgtagaaaagatcaaaggatcttcttgagatcctttttttctgcgcgtaatctgctgcttgcaaacaaaaaaaccaccgctaccagcggtggtttgtttgccggatcaagagctaccaactctttttccgaaggtaactggcttcagcagagcgcagataccaaatactgtccttctagtgtagccgtagttaggccaccacttcaagaactctgtagcaccgcctacatacctcgctctgctaatcctgttaccagtggctgctgccagtggcgataagtcgtgtcttaccgggttggactcaagacgatagttaccggataaggcgcagcggtcgggctgaacggggggttcgtgcacacagcccagcttggagcgaacgacctacaccgaactgagatacctacagcgtgagctatgagaaagcgccacgcttcccgaagggagaaaggcggacaggtatccggtaagcggcagggtcggaacaggagagcgcacgagggagcttccagggggaaacgcctggtatctttatagtcctgtcgggtttcgccacctctgacttgagcgtcgatttttgtgatgctcgtcaggggggcggagcctatggaaaaacgccagcaacgcggcctttttacggttcctggccttttgctggccttttgctcacatgttctttcctgcgttatcccctgattctgtggataaccgtattaccgcctttgagtgagctgataccgctcgccgcagccgaacgaccgagcgcagcgagtcagtgagcgaggaagcggaagagcgcccaatacgcaaaccgcctctccccgcgcgttggccgattcattaatgcagctgtggaatgtgtgtcagttagggtgtggaaagtccccaggctccccagcaggcagaagtatgcaaagcatgcatctcaattagtcagcaaccaggtgtggaaagtccccaggctccccagcaggcagaagtatgcaaagcatgcatctcaattagtcagcaaccatagtcccgcccctaactccgcccatcccgcccctaactccgcccagttccgcccattctccgccccatggctgactaattttttttatttatgcagaggccgaggccgcctcggcctctgagctattccagaagtagtgaggaggcttttttggaggcctaggcttttgcaaaaagcttggacacaagacaggcttgcgagatatgtttgagaataccactttatcccgcgtcagggagaggcagtgcgtaaaaagacgcggactcatgtgaaatactggtttttagtgcgccagatctctataatctcgcgcaacctattttcccctcgaacactttttaagccgtagataaacaggctgggacacttcacatgagcgaaaaatacatcgtcacctgggacatgttgcagatccatgcacgtaaactcgcaagccgactgatgccttctgaacaatggaaaggcattattgccgtaagccgtggcggtctgtaccgggtgcgttactggcgcgtgaactgggtattcgtcatgtcgataccgtttgtatttccagctacgatcacgacaaccagcgcgagcttaaagtgctgaaacgcgcagaaggcgatggcgaaggcttcatcgttattgatgacctggtggataccggtggtactgcggttgcgattcgtgaaatgtatccaaaagcgcactttgtcaccatcttcgcaaaaccggctggtcgtccgctggttgatgactatgttgttgatatcccgcaagatacctggattgaacagccgtgggatatgggcgtcgtattcgtcccgccaatctccggtcgctaatcttttcaacgcctggcactgccgggcgttgttctttttaacttcaggcgggttacaatagtttccagtaagtattctggaggctgcatccatgacacaggcaaacctgagcgaaaccctgttcaaaccccgctttaaacatcctgaaacctcgacgctagtccgccgctttaatcacggcgcacaaccgcctgtgcagtcggcccttgatggtaaaaccatccctcactggtatcgcatgattaaccgtctgatgtggatctggcgcggcattgacccacgcgaaatcctcgacgtccaggcacgtattgtgatgagcgatgccgaacgtaccgacgatgatttatacgatacggtgattggctaccgtggcggcaactggatttatgagtgggccccggatctttgtgaaggaaccttacttctgtggtgtgacataattggacaaactacctacagagatttaaagctctaaggtaaatataaaatttttaagtgtataatgtgttaaactactgattctaattgtttgtgtattttagattccaacctatggaactgatgaatgggagcagtggtggaatgcctttaatgaggaaaacctgttttgctcagaagaaatgccatctagtgatgatgaggctactgctgactctcaacattctactcctccaaaaaagaagagaaaggtagaagaccccaaggactttccttcagaattgctaagttttttgagtcatgctgtgtttagtaatagaactcttgcttgctttgctatttacaccacaaaggaaaaagctgcactgctatacaagaaaattatggaaaaatattctgtaacctttataagtaggcataacagttataatcataacatactgttttttcttactccacacaggcatagagtgtctgctattaataactatgctcaaaaattgtgtacctttagctttttaatttgtaaaggggttaataaggaatatttgatgtatagtgccttgactagagatcataatcagccataccacatttgtagaggttttacttgctttaaaaaacctcccacacctccccctgaacctgaaacataaaatgaatgcaattgttgttgttaacttgtttattgcagcttataatggttacaaataaagcaatagcatcacaaatttcacaaataaagcatttttttcactgcattctagttgtggtttgtccaaactcatcaatgtatcttatcatgtctggatcaactggataactcaagctaaccaaaatcatcccaaacttcccaccccataccctattaccactgccaattacctagtggtttcatttactctaaacctgtgattcctctgaattattttcattttaaagaaattgtatttgttaaatatgtactacaaacttagtagttggaagggctaattcactcccaaagaagacaagatatccttgatctgtggatctaccacacacaaggctacttccctgattagcagaactacacaccagggccaggggtcagatatccactgacctttggatggtgctacaagctagtaccagttgagccagataaggtagaagaggccaataaaggagagaacaccagcttgttacaccctgtgagcctgcatgggatggatgacccggagagagaagtgttagagtggaggtttgacagccgcctagcatttcatcacgtggcccgagagctgcatccggagtacttcaagaactgctgatatcgagcttgctacaagggactttccgctggggactttccagggaggcgtggcctgggcgggactggggagtggcgagccctcagatcctgcatataagcagctgctttttgcctgtactgggtctctctggttagaccagatctgagcctgggagctctctggctaactagggaacccactgcttaagcctcaataaagcttgccttgagtgcttcaagtagtgtgtgcccgtctgttgtgtgactctggtaactagagatccctcagacccttttagtcagtgtggaaaatctctagcagtggcgcccgaacagggacttgaaagcgaaagggaaaccagaggagctctctcgacgcaggactcggcttgctgaagcgcgcacggcaagaggcgaggggcggcgactggtgagtacgccaaaaattttgactagcggaggctagaaggagagagatgggtgcgagagcgtcagtattaagcgggggagaattagatcgcgatgggaaaaaattcggttaaggccagggggaaagaaaaaatataaattaaaacatatagtatgggcaagcagggagctagaacgattcgcagttaatcctggcctgttagaaacatcagaaggctgtagacaaatactgggacagctacaaccatcccttcagacaggatcagaagaacttagatcattatataatacagtagcaaccctctattgtgtgcatcaaaggatagagataaaagacaccaaggaagctttagacaagatagaggaagagcaaaacaaaagtaagaccaccgcacagcaagcggccggtgatcttcagacctggacgatatatatgagggacaattggagaagtgaattatataaatataaagtagtaaaaattgaaccattaggagtagcacccaccaaggcaaagagaagagtggtgcagagagaaaaaagagcagtgggaataggagctttgttccttgggttcttgggagcagcaggaagcactatgggcgcagcgtcaatgacgctgacggtacaggccagacaattattgtctggtatagtgcagcagcagaacaatttgctgagggctattgaggcgcaacagcatctgttgcaactcacagtctggggcatcaagcagctccaggcaagaatcctggctgtggaaagatacctaaaggatcaacagctcctggggatttggggttgctctggaaaactcatttgcaccactgctgtgccttggaatgctagttggagtaataaatctctggaacagatttggaatcacacgacctggatggagtgggacagagaaattaacaattacacaagcttaatacactccttaattgaagaatcgcaaaaccagcaagaaaagaatgaacaagaattattggaattagataaatgggcaagtttgtggaattggtttaacataacaaattggctgtggtatataaaattattcataatgatagtaggaggcttggtaggtttaagaatagtttttgctgtactttctatagtgaatagagttaggcagggatattcaccattatcgtttcagacccacctcccaaccccgaggggacccgacaggcccgaaggaatagaagaagaaggtggagagagagacagagacagatccattcgattagtgaacggatctcgacggtcgccaaatggcagtattcatccacaattttaaaagaaaaggggggattggggggtacagtgcaggggaaagaatagtagacataatagcaacagacatacaaactaaagaattacaaaaacaaattacaaaaattcaaaattttcgggtttattacagggacagcagagatccagtttggatcgataagcttgatatcgaattgggtaggggaggcgcttttcccaaggcagtctggagcatgcgctttagcagccccgctgggcacttggcgctacacaagtggcctctggcctcgcacacattccacatccaccggtaggcgccaaccggctccgttctttggtggccccttcgcgccaccttctactcctcccctagtcaggaagttcccccccgccccgcagctcgcgtcgtgcaggacgtgacaaatggaagtagcacgtctcactagtctcgtgcagatggacagcaccgctgagcaatggaagcgggtaggcctttggggcagcggccaatagcagctttgctccttcgctttctgggctcagaggctgggaaggggtgggtccgggggcgggctcaggggcgggctcaggggcggggcgggcgcccgaaggtcctccggaggcccggcattctgcacgcttcaaaagcgcacgtctgccgcgctgttctcctcttcctcatctccgggcctttcgatggctcttccagtgactgctcttctcctcccgcttgcgctgctgttgcatgcggctcggccggagcaaaagctgatttcagaagaggacttggatatccagatgacacagaccacttcatctctttctgctagcctgggggatcgggtcacaataagctgtcgcgcatcccaagacataagcaaatatctgaattggtatcaacagaaacccgatggaactgtgaaacttctcatctaccatacgagcagactgcattctggggttcctagccgcttttcagggtctggatctggaacggactattcacttaccatatctaatttggaacaagaagacatcgcgacctatttctgtcagcaaggcaatacgctcccttatacttttggagggggaacgaagttggagatcacaggtggaggcggcagtggcgggggaggatctggtggaggtggttctgaggtcaagctgcaggagagtggtcccgggctggtagccccgagccagagtctgtctgttacttgcactgtgtcaggcgtgagtctcccagactatggtgtatcatggattcgacagccgccccggaaaggacttgagtggctcggagtgatctggggatccgaaacgacgtactacaatagcgcgctcaaaagccggctgaccatcattaaggataactctaaaagccaggtgttcttgaaaatgaattccttgcagacagatgatacggcgatctattactgtgccaagcactactactatggaggcagctatgccatggattattggggtcaaggcacttctgtgacagtgagcagtgccgcagctattgaagtgatgtacccgcctccgtatcttgataatgagaaatctaacggaaccataatacacgtgaaaggcaaacatttgtgtccgtctcctctgttccccgggcctagtaaaccgttttgggtactggtggtggtaggcggagtacttgcatgttactcactcctcgttaccgtcgcattcattatcttctgggtacggagcaagagatctcggctgcttcatagcgattatatgaatatgacacccagacgcccaggtcctactaggaaacattaccagccgtatgcgccgccgagggacttcgccgcatacagatctcgcgtgaagttctcaagatctgccgatgcaccggcttatcagcagggacaaaaccaactgtataatgagctgaacctggggcggagggaggagtatgatgtcctggacaagcgaagagggcgagaccccgaaatgggaggcaagcctcaacggcggaagaacccacaagagggcctgtataacgagcttcaaaaggacaaaatggcggaagcgtatagcgagatcggaatgaagggcgaacgaaggagagggaaaggtcacgatgggctctaccaggggctcagcacggcaacaaaagacacatatgacgcattgcatatgcaggcgctgccaccgagatgactcacgcgtcaagtggagcaaggcaggtggacagtggatccttgacttgcggccgcaactcccacctgcaacatgcgtgactgactgaggccgcgactctagagtcgacctgcaggcatgcaagcttgatatcaagcttatcgataatcaacctctggattacaaaatttgtgaaagattgactggtattcttaactatgttgctccttttacgctatgtggatacgctgctttaatgcctttgtatcatgctattgcttcccgtatggctttcattttctcctccttgtataaatcctggttgctgtctctttatgaggagttgtggcccgttgtcaggcaacgtggcgtggtgtgcactgtgtttgctgacgcaacccccactggttggggcattgccaccacctgtcagctcctttccgggactttcgctttccccctccctattgccacggcggaactcatcgccgcctgccttgcccgctgctggacaggggctcggctgttgggcactgacaattccgtggtgttgtcggggaaatcatcgtcctttccttggctgctcgcctgtgttgccacctggattctgcgcgggacgtccttctgctacgtcccttcggccctcaatccagcggaccttccttcccgcggcctgctgccggctctgcggcctcttccgcgtcttcgccttcgccctcagacgagtcggatctccctttgggccgcctccccgcat

SEQ ID NO: 10 - DNA, 12536 bp, artificial
  pWPI pmei mAnti cd19 1D3 myc hinge cd28 cd3zeta
ttggaagggctaattcactcccaaagaagacaagatatccttgatctgtggatctaccacacacaaggctacttccctgattagcagaactacacaccagggccaggggtcagatatccactgacctttggatggtgctacaagctagtaccagttgagccagataaggtagaagaggccaataaaggagagaacaccagcttgttacaccctgtgagcctgcatgggatggatgacccggagagagaagtgttagagtggaggtttgacagccgcctagcatttcatcacgtggcccgagagctgcatccggagtacttcaagaactgctgatatcgagcttgctacaagggactttccgctggggactttccagggaggcgtggcctgggcgggactggggagtggcgagccctcagatcctgcatataagcagctgctttttgcctgtactgggtctctctggttagaccagatctgagcctgggagctctctggctaactagggaacccactgcttaagcctcaataaagcttgccttgagtgcttcaagtagtgtgtgcccgtctgttgtgtgactctggtaactagagatccctcagacccttttagtcagtgtggaaaatctctagcagtggcgcccgaacagggacttgaaagcgaaagggaaaccagaggagctctctcgacgcaggactcggcttgctgaagcgcgcacggcaagaggcgaggggcggcgactggtgagtacgccaaaaattttgactagcggaggctagaaggagagagatgggtgcgagagcgtcagtattaagcgggggagaattagatcgcgatgggaaaaaattcggttaaggccagggggaaagaaaaaatataaattaaaacatatagtatgggcaagcagggagctagaacgattcgcagttaatcctggcctgttagaaacatcagaaggctgtagacaaatactgggacagctacaaccatcccttcagacaggatcagaagaacttagatcattatataatacagtagcaaccctctattgtgtgcatcaaaggatagagataaaagacaccaaggaagctttagacaagatagaggaagagcaaaacaaaagtaagaccaccgcacagcaagcggccgctgatcttcagacctggaggaggagatatgagggacaattggagaagtgaattatataaatataaagtagtaaaaattgaaccattaggagtagcacccaccaaggcaaagagaagagtggtgcagagagaaaaaagagcagtgggaataggagctttgttccttgggttcttgggagcagcaggaagcactatgggcgcagcgtcaatgacgctgacggtacaggccagacaattattgtctggtatagtgcagcagcagaacaatttgctgagggctattgaggcgcaacagcatctgttgcaactcacagtctggggcatcaagcagctccaggcaagaatcctggctgtggaaagatacctaaaggatcaacagctcctggggatttggggttgctctggaaaactcatttgcaccactgctgtgccttggaatgctagttggagtaataaatctctggaacagatttggaatcacacgacctggatggagtgggacagagaaattaacaattacacaagcttaatacactccttaattgaagaatcgcaaaaccagcaagaaaagaatgaacaagaattattggaattagataaatgggcaagtttgtggaattggtttaacataacaaattggctgtggtatataaaattattcataatgatagtaggaggcttggtaggtttaagaatagtttttgctgtactttctatagtgaatagagttaggcagggatattcaccattatcgtttcagacccacctcccaaccccgaggggacccgacaggcccgaaggaatagaagaagaaggtggagagagagacagagacagatccattcgattagtgaacggatctcgacggtatcgatgtcgacgataagctttgcaaagatggataaagttttaaacagagaggaatctttgcagctaatggaccttctaggtcttgaaaggagtgggaattggctccggtgcccgtcagtgggcagagcgcacatcgcccacagtccccgagaagttggggggaggggtcggcaattgaaccggtgcctagagaaggtggcgcggggtaaactgggaaagtgatgtcgtgtactggctccgcctttttcccgagggtgggggagaaccgtatataagtgcagtagtcgccgtgaacgttctttttcgcaacgggtttgccgccagaacacaggtaagtgccgtgtgtggttcccgcgggcctggcctctttacgggttatggcccttgcgtgccttgaattacttccactggctgcagtacgtgattcttgatcccgagcttcgggttggaagtgggtgggagagttcgaggccttgcgcttaaggagccccttcgcctcgtgcttgagttgaggcctggcctgggcgctggggccgccgcgtgcgaatctggtggcaccttcgcgcctgtctcgctgctttcgataagtctctagccatttaaaatttttgatgacctgctgcgacgctttttttctggcaagatagtcttgtaaatgcgggccaagatctgcacactggtatttcggtttttggggccgcgggcggcgacggggcccgtgcgtcccagcgcacatgttcggcgaggcggggcctgcgagcgcggccaccgagaatcggacgggggtagtctcaagctggccggcctgctctggtgcctggcctcgcgccgccgtgtatcgccccgccctgggcggcaaggctggcccggtcggcaccagttgcgtgagcggaaagatggccgcttcccggccctgctgcagggagctcaaaatggaggacgcggcgctcgggagagcgggcgggtgagtcacccacacaaaggaaaagggcctttccgtcctcagccgtcgcttcatgtgactccacggagtaccgggcgccgtccaggcacctcgattagttctcgagcttttggagtacgtcgtctttaggttggggggaggggttttatgcgatggagtttccccacactgagtgggtggagactgaagttaggccagcttggcacttgatgtaattctccttggaatttgccctttttgagtttggatcttggttcattctcaagcctcagacagtggttcaaagtttttttcttccatttcaggtgtcgtgaggaatttcgacatttaaatttaattaatctcgacggtatcggttaacttttaaaagaaaaggggggattggggggtacagtgcaggggaaagaatagtagacataatagcaacagacatacaaactaaagaattacaaaaacaaattacaaaaattcaaaattttatcgatcacgagactagcctcgaggtttatgggggttcccacccagctgttggggttgctgctcctctggatcactgatgccatctgcgaacagaagctcatttctgaagaagatctggacatacagatgacccagagtcctgccagcttgtccacatccctcggagagaccgtgacaattcaatgccaggcctctgaggacatatattctggattggcttggtaccagcaaaagccaggtaaaagtcctcagttgttgatatacggcgcttctgatttgcaagacggggtgccctcacgatttagcgggtctggaagtggcactcagtacagtctgaagattacttcaatgcaaacagaagacgagggtgtgtatttttgccaacaggggctgacctacccaaggacattcgggggcggtacaaagcttgaacttaagggcggcggtgggtctggaggtggtggatctggcggagggggaagtgaggtacagctgcaacagtccggcgccgaactcgttcgccctggaacctcagtcaaattgtcatgcaaggtgagtggcgacacaataaccttttactatatgcacttcgttaaacagaggccaggtcaaggtctggaatggataggcagaattgatccagaagatgagtccaccaaatactcagaaaagttcaaaaacaaagccactcttactgccgacacctcaagcaacacagcatatcttaagctcagttcacttaccagcgaagacaccgccacctatttttgtatttatggtggctattactttgactactgggggcaaggtgttatggtaacagtttcttccattgaattcatgtatccacccccctatttggataatgaacgatctaatgggactataatacatatcaaggaaaagcatctgtgtcatacccaaagttcccctaagcttttctgggccctcgtcgttgtggcaggagtgcttttttgctatggattgttggttactgtggctctctgcgtcatttggacaaatagtaggaggaatcgggggggacaatctgattacatgaacatgacaccacggaggccaggccttaccagaaagccctaccaaccttatgcaccagcacgagacttcgccgcatacaggccaagggctaagttttcccgcagcgccgaaaccgcagccaacctccaagatcctaatcagctctataacgaattgaatcttggccgcagagaggagtacgacgtacttgagaaaaagagagctagggaccctgaaatgggtgggaagcaacagcgaagaaggaacccacaggaaggggtgtataatgcccttcaaaaggataaaatggcagaggcatacagtgaaatcggaaccaagggggagagacgcagagggaaaggccatgacggcctttatcagggtttgtcaactgctactaaagacacttatgatgccttgcatatgcaaactctcgcacccagatgaaaactacgggctgcaggaattccgcccccccccccctaacgttactggccgaagccgcttggaataaggccggtgtgcgtttgtctatatgttattttccaccatattgccgtcttttggcaatgtgagggcccggaaacctggccctgtcttcttgacgagcattcctaggggtctttcccctctcgccaaaggaatgcaaggtctgttgaatgtcgtgaaggaagcagttcctctggaagcttcttgaagacaaacaacgtctgtagcgaccctttgcaggcagcggaaccccccacctggcgacaggtgcctctgcggccaaaagccacgtgtataagatacacctgcaaaggcggcacaaccccagtgccacgttgtgagttggatagttgtggaaagagtcaaatggctctcctcaagcgtattcaacaaggggctgaaggatgcccagaaggtaccccattgtatgggatctgatctggggcctcggtgcacatgctttacatgtgtttagtcgaggttaaaaaacgtctaggccccccgaaccacggggacgtggttttcctttgaaaaacacgatgataataccatggtgagcaagggcgaggagctgttcaccggggtggtgcccatcctggtcgagctggacggcgacgtaaacggccacaagttcagcgtgtccggcgagggcgagggcgatgccacctacggcaagctgaccctgaagttcatctgcaccaccggcaagctgcccgtgccctggcccaccctcgtgaccaccctgacctacggcgtgcagtgcttcagccgctaccccgaccacatgaagcagcacgacttcttcaagtccgccatgcccgaaggctacgtccaggagcgcaccatcttcttcaaggacgacggcaactacaagacccgcgccgaggtgaagttcgagggcgacaccctggtgaaccgcatcgagctgaagggcatcgacttcaaggaggacggcaacatcctggggcacaagctggagtacaactacaacagccacaacgtctatatcatggccgacaagcagaagaacggcatcaaggtgaacttcaagatccgccacaacatcgaggacggcagcgtgcagctcgccgaccactaccagcagaacacccccatcggcgacggccccgtgctgctgcccgacaaccactacctgagcacccagtccgccctgagcaaagaccccaacgagaagcgcgatcacatggtcctgctggagttcgtgaccgccgccgggatcactctcggcatggacgagctgtacaagtccggactcagatctcgactagctagtagctagctagctagtcgagctcaagcttcgaattcgatatcaagcttatcgcgataccgtcgacctcgagggaattccgataatcaacctctggattacaaaatttgtgaaagattgactggtattcttaactatgttgctccttttacgctatgtggatacgctgctttaatgcctttgtatcatgctattgcttcccgtatggctttcattttctcctccttgtataaatcctggttgctgtctctttatgaggagttgtggcccgttgtcaggcaacgtggcgtggtgtgcactgtgtttgctgacgcaacccccactggttggggcattgccaccacctgtcagctcctttccgggactttcgctttccccctccctattgccacggcggaactcatcgccgcctgccttgcccgctgctggacaggggctcggctgttgggcactgacaattccgtggtgttgtcggggaagctgacgtcctttccatggctgctcgcctgtgttgccacctggattctgcgcgggacgtccttctgctacgtcccttcggccctcaatccagcggaccttccttcccgcggcctgctgccggctctgcggcctcttccgcgtcttcgccttcgccctcagacgagtcggatctccctttgggccgcctccccgcatcgggaattcgagctcggtacctttaagaccaatgacttacaaggcagctgtagatcttagccactttttaaaagaaaaggggggactggaagggctaattcactcccaacgaagacaagatgggatcaattcaccatgggaataacttcgtatagcatacattatacgaagttatgctgctttttgcttgtactgggtctctctggttagaccagatctgagcctgggagctctctggctaactagggaacccactgcttaagcctcaataaagcttgccttgagtgcttcaagtagtgtgtgcccgtctgttgtgtgactctggtaactagagatccctcagacccttttagtcagtgtggaaaatctctagcagcatctagaattaattccgtgtattctatagtgtcacctaaatcgtatgtgtatgatacataaggttatgtattaattgtagccgcgttctaacgacaatatgtacaagcctaattgtgtagcatctggcttactgaagcagaccctatcatctctctcgtaaactgccgtcagagtcggtttggttggacgaaccttctgagtttctggtaacgccgtcccgcacccggaaatggtcagcgaaccaatcagcagggtcatcgctagccagatcctctacgccggacgcatcgtggccggcatcaccggcgccacaggtgcggttgctggcgcctatatcgccgacatcaccgatggggaagatcgggctcgccacttcgggctcatgagcgcttgtttcggcgtgggtatggtggcaggccccgtggccgggggactgttgggcgccatctccttgcatgcaccattccttgcggcggcggtgctcaacggcctcaacctactactgggctgcttcctaatgcaggagtcgcataagggagagcgtcgaatggtgcactctcagtacaatctgctctgatgccgcatagttaagccagccccgacacccgccaacacccgctgacgcgccctgacgggcttgtctgctcccggcatccgcttacagacaagctgtgaccgtctccgggagctgcatgtgtcagaggttttcaccgtcatcaccgaaacgcgcgagacgaaagggcctcgtgatacgcctatttttataggttaatgtcatgataataatggtttcttagacgtcaggtggcacttttcggggaaatgtgcgcggaacccctatttgtttatttttctaaatacattcaaatatgtatccgctcatgagacaataaccctgataaatgcttcaataatattgaaaaaggaagagtatgagtattcaacatttccgtgtcgcccttattcccttttttgcggcattttgccttcctgtttttgctcacccagaaacgctggtgaaagtaaaagatgctgaagatcagttgggtgcacgagtgggttacatcgaactggatctcaacagcggtaagatccttgagagttttcgccccgaagaacgttttccaatgatgagcacttttaaagttctgctatgtggcgcggtattatcccgtattgacgccgggcaagagcaactcggtcgccgcatacactattctcagaatgacttggttgagtactcaccagtcacagaaaagcatcttacggatggcatgacagtaagagaattatgcagtgctgccataaccatgagtgataacactgcggccaacttacttctgacaacgatcggaggaccgaaggagctaaccgcttttttgcacaacatgggggatcatgtaactcgccttgatcgttgggaaccggagctgaatgaagccataccaaacgacgagcgtgacaccacgatgcctgtagcaatggcaacaacgttgcgcaaactattaactggcgaactacttactctagcttcccggcaacaattaatagactggatggaggcggataaagttgcaggaccacttctgcgctcggcccttccggctggctggtttattgctgataaatctggagccggtgagcgtgggtctcgcggtatcattgcagcactggggccagatggtaagccctcccgtatcgtagttatctacacgacggggagtcaggcaactatggatgaacgaaatagacagatcgctgagataggtgcctcactgattaagcattggtaactgtcagaccaagtttactcatatatactttagattgatttaaaacttcatttttaatttaaaaggatctaggtgaagatcctttttgataatctcatgaccaaaatcccttaacgtgagttttcgttccactgagcgtcagaccccgtagaaaagatcaaaggatcttcttgagatcctttttttctgcgcgtaatctgctgcttgcaaacaaaaaaaccaccgctaccagcggtggtttgtttgccggatcaagagctaccaactctttttccgaaggtaactggcttcagcagagcgcagataccaaatactgtccttctagtgtagccgtagttaggccaccacttcaagaactctgtagcaccgcctacatacctcgctctgctaatcctgttaccagtggctgctgccagtggcgataagtcgtgtcttaccgggttggactcaagacgatagttaccggataaggcgcagcggtcgggctgaacggggggttcgtgcacacagcccagcttggagcgaacgacctacaccgaactgagatacctacagcgtgagcattgagaaagcgccacgcttcccgaagggagaaaggcggacaggtatccggtaagcggcagggtcggaacaggagagcgcacgagggagcttccagggggaaacgcctggtatctttatagtcctgtcgggtttcgccacctctgacttgagcgtcgatttttgtgatgctcgtcaggggggcggagcctatggaaaaacgccagcaacgcggcctttttacggttcctggccttttgctggccttttgctcacatgttctttcctgcgttatcccctgattctgtggataaccgtattaccgcctttgagtgagctgataccgctcgccgcagccgaacgaccgagcgcagcgagtcagtgagcgaggaagcggaagagcgcccaatacgcaaaccgcctctccccgcgcgttggccgattcattaatgcagctgtggaatgtgtgtcagttagggtgtggaaagtccccaggctccccagcaggcagaagtatgcaaagcatgcatctcaattagtcagcaaccaggtgtggaaagtccccaggctccccagcaggcagaagtatgcaaagcatgcatctcaattagtcagcaaccatagtcccgcccctaactccgcccatcccgcccctaactccgcccagttccgcccattctccgccccatggctgactaattttttttatttatgcagaggccgaggccgcctcggcctctgagctattccagaagtagtgaggaggcttttttggaggcctaggcttttgcaaaaagcttggacacaagacaggcttgcgagatatgtttgagaataccactttatcccgcgtcagggagaggcagtgcgtaaaaagacgcggactcatgtgaaatactggtttttagtgcgccagatctctataatctcgcgcaacctattttcccctcgaacactttttaagccgtagataaacaggctgggacacttcacatgagcgaaaaatacatcgtcacctgggacatgttgcagatccatgcacgtaaactcgcaagccgactgatgccttctgaacaatggaaaggcattattgccgtaagccgtggcggtctgtaccgggtgcgttactggcgcgtgaactgggtattcgtcatgtcgataccgtttgtatttccagctacgatcacgacaaccagcgcgagcttaaagtgctgaaacgcgcagaaggcgatggcgaaggcttcatcgttattgatgacctggtggataccggtggtactgcggttgcgattcgtgaaatgtatccaaaagcgcactttgtcaccatcttcgcaaaaccggctggtcgtccgctggttgatgactatgttgttgatatcccgcaagatacctggattgaacagccgtgggatatgggcgtcgtattcgtcccgccaatctccggtcgctaatcttttcaacgcctggcactgccgggcgttgttctttttaacttcaggcgggttacaatagtttccagtaagtattctggaggctgcatccatgacacaggcaaacctgagcgaaaccctgttcaaaccccgctttaaacatcctgaaacctcgacgctagtccgccgctttaatcacggcgcacaaccgcctgtgcagtcggcccttgatggtaaaaccatccctcactggtatcgcatgattaaccgtctgatgtggatctggcgcggcattgacccacgcgaaatcctcgacgtccaggcacgtattgtgatgagcgatgccgaacgtaccgacgatgatttatacgatacggtgattggctaccgtggcggcaactggatttatgagtgggccccggatctttgtgaaggaaccttacttctgtggtgtgacataattggacaaactacctacagagatttaaagctctaaggtaaatataaaatttttaagtgtataatgtgttaaactactgattctaattgtttgtgtattttagattccaacctatggaactgatgaatgggagcagtggtggaatgcctttaatgaggaaaacctgttttgctcagaagaaatgccatctagtgatgatgaggctactgctgactctcaacattctactcctccaaaaaagaagagaaaggtagaagaccccaaggactttccttcagaattgctaagttttttgagtcatgctgtgtttagtaatagaactcttgcttgctttgctatttacaccacaaaggaaaaagctgcactgctatacaagaaaattatggaaaaatattctgtaacctttataagtaggcataacagttataatcataacatactgttttttcttactccacacaggcatagagtgtctgctattaataactatgctcaaaaattgtgtacctttagctttttaatttgtaaaggggttaataaggaatatttgatgtatagtgccttgactagagatcataatcagccataccacatttgtagaggttttacttgctttaaaaaacctcccacacctccccctgaacctgaaacataaaatgaatgcaattgttgttgttaacttgtttattgcagcttataatggttacaaataaagcaatagcatcacaaatttcacaaataaagcatttttttcactgcattctagttgtggtttgtccaaactcatcaatgtatcttatcatgtctggatcaactggataactcaagctaaccaaaatcatcccaaacttcccaccccataccctattaccactgccaattacctagtggtttcatttactctaaacctgtgattcctctgaattattttcattttaaagaaattgtatttgttaaatatgtactacaaacttagtag

SEQ ID NO: 11 - protein, 365 aa, artificial
  FKBP-1SG-FR with GPI anchor amino acid sequence
MTTQLLLLLVWVAVVGEAQTGVQVETISPGDGRTFPKRGQTCVVHYTGMLEDGKKFDSSRDRNKPFKFMLGKQEVIRGWEEGVAQMSVGQRAKLTISPDYAYGATGHPGIIPPHATLVFDVELLKLESGGGSRIAWARTELLNVCMNAKHHKEKPGPEDKLHEQCRPWRKNACCSTNTSQEAHKDVSYLYRFNWNHCGEMAPACKRHFIQDTCLYECSPNLGPWIQQVDQSWRKERVLNVPLCKEDCEQWWEDCRTSYTCKSNWHKGWNWTSGFNKCAVGAACQPFHFYFPTPTVLCNEIWTHSYKVSNYSRGSGRCIQMWFDPAQGNPNEEVARFYAAAMSGAGPWAAWPFLLSLALMLLWLLS

SEQ ID NO: 12 - protein, 375 aa, artificial
  FKBP-3SG-FR with GPI anchor amino acid sequence:
MTTQLLLLLVWVAVVGEAQTGVQVETISPGDGRTFPKRGQTCVVHYTGMLEDGKKFDSSRDRNKPFKFMLGKQEVIRGWEEGVAQMSVGQRAKLTISPDYAYGATGHPGIIPPHATLVFDVELLKLEGGGGSGGGGSGGGGSRIAWARTELLNVCMNAKHHKEKPGPEDKLHEQCRPWRKNACCSTNTSQEAHKDVSYLYRFNWNHCGEMAPACKRHFIQDTCLYECSPNLGPWIQQVDQSWRKERVLNVPLCKEDCEQWWEDCRTSYTCKSNWHKGWNWTSGFNKCAVGAACQPFHFYFPTPTVLCNEIWTHSYKVSNYSRGSGRCIQMWFDPAQGNPNEEVARFYAAAMSGAGPWAAWPFLLSLALMLLWLLS

SEQ ID NO: 13 - protein, 513 aa, artificial
  4M5.3-FR with GPI anchor amino acid sequence
MALPVTALLLPLALLLHAARPDVVMTQTPLSLPVSLGDQASISCRSSQSLVHSNGNTYLRWYLQKPGQSPKVLIYKVSNRVSGVPDRFSGSGSGTDFTLKINRVEAEDLGVYFCSQSTHVPWTFGGGTKLEIKSSADDAKKDAAKKDDAKKDDAKKDGGVKLDETGGGLVQPGGAMKLSCVTSGFTFGHYWMNWVRQSPEKGLEWVAQFRNKPYNYETYYSDSVKGRFTISRDDSKSSVYLQMNNLRVEDTGIYYCTGASYGMEYLGQGTSVTVSSGGGSRIAWARTELLNVCMNAKHHKEKPGPEDKLHEQCRPWRKNACCSTNTSQEAHKDVSYLYRFNWNHCGEMAPACKRHFIQDTCLYECSPNLGPWIQQVDQSWRKERVLNVPLCKEDCEQWWEDCRTSYTCKSNWHKGWNWTSGFNKCAVGAACQPFHFYFPTPTVLCNEIWTHSYKVSNYSRGSGRCIQMWFDPAQGNPNEEVARFYAAAMSGAGPWAAWPFLLSLALMLLWLLS

SEQ ID NO: 14 - protein, 895 aa, artificial
  FMC63-T2A-FKBP3SGFR
MALPVTALLLPLALLLHAARPEQKLISEEDLDIQMTQTTSSLSASLGDRVTISCRASQDISKYLNWYQQKPDGTVKLLIYHTSRLHSGVPSRFSGSGSGTDYSLTISNLEQEDIATYFCQQGNTLPYTFGGGTKLEITGGGGSGGGGSGGGGSEVKLQESGPGLVAPSQSLSVTCTVSGVSLPDYGVSWIRQPPRKGLEWLGVIWGSETTYYNSALKSRLTIIKDNSKSQVFLKMNSLQTDDTAIYYCAKHYYYGGSYAMDYWGQGTSVTVSSAAAIEVMYPPPYLDNEKSNGTIIHVKGKHLCPSPLFPGPSKPFWVLVVVGGVLACYSLLVTVAFIIFWVRSKRSRLLHSDYMNMTPRRPGPTRKHYQPYAPPRDFAAYRSRVKFSRSADAPAYQQGQNQLYNELNLGRREEYDVLDKRRGRDPEMGGKPRRKNPQEGLYNELQKDKMAEAYSEIGMKGERRRGKGHDGLYQGLSTATKDTYDALHMQALPPRGSGEGRGSLLTCGDVEENPGPMAQRMTTQLLLLLVWVAVVGEAQTGVQVETISPGDGRTFPKRGQTCVVHYTGMLEDGKKFDSSRDRNKPFKFMLGKQEVIRGWEEGVAQMSVGQRAKLTISPDYAYGATGHPGIIPPHATLVFDVELLKLEGGGGSGGGGSGGGGSRIAWARTELLNVCMNAKHHKEKPGPEDKLHEQCRPWRKNACCSTNTSQEAHKDVSYLYRFNWNHCGEMAPACKRHFIQDTCLYECSPNLGPWIQQVDQSWRKERVLNVPLCKEDCEQWWEDCRTSYTCKSNWHKGWNWTSGFNKCAVGAACQPFHFYFPTPTVLCNEIWTHSYKVSNYSRGSGRCIQMWFDPAQGNPNEEVARFYAAAMSGAGPWAAWPFLLSLALMLLWLLS

SEQ ID NO: 15 - protein, 1029 aa, artificial
  FMC63-T2A-4M5.3SGFR
MALPVTALLLPLALLLHAARPEQKLISEEDLDIQMTQTTSSLSASLGDRVTISCRASQDISKYLNWYQQKPDGTVKLLIYHTSRLHSGVPSRFSGSGSGTDYSLTISNLEQEDIATYFCQQGNTLPYTFGGGTKLEITGGGGSGGGGSGGGGSEVKLQESGPGLVAPSQSLSVTCTVSGVSLPDYGVSWIRQPPRKGLEWLGVIWGSETTYYNSALKSRLTIIKDNSKSQVFLKMNSLQTDDTAIYYCAKHYYYGGSYAMDYWGQGTSVTVSSAAAIEVMYPPPYLDNEKSNGTIIHVKGKHLCPSPLFPGPSKPFWVLVVVGGVLACYSLLVTVAFIIFWVRSKRSRLLHSDYMNMTPRRPGPTRKHYQPYAPPRDFAAYRSRVKFSRSADAPAYQQGQNQLYNELNLGRREEYDVLDKRRGRDPEMGGKPRRKNPQEGLYNELQKDKMAEAYSEIGMKGERRRGKGHDGLYQGLSTATKDTYDALHMQALPPRGSGEGRGSLLTCGDVEENPGPMALPVTALLLPLALLLHAARPDVVMTQTPLSLPVSLGDQASISCRSSQSLVHSNGNTYLRWYLQKPGQSPKVLIYKVSNRVSGVPDRFSGSGSGTDFTLKINRVEAEDLGVYFCSQSTHVPWTFGGGTKLEIKSSADDAKKDAAKKDDAKKDDAKKDGGVKLDETGGGLVQPGGAMKLSCVTSGFTFGHYWMNWVRQSPEKGLEWVAQFRNKPYNYETYYSDSVKGRFTISRDDSKSSVYLQMNNLRVEDTGIYYCTGASYGMEYLGQGTSVTVSSGGGSRIAWARTELLNVCMNAKHHKEKPGPEDKLHEQCRPWRKNACCSTNTSQEAHKDVSYLYRFNWNHCGEMAPACKRHFIQDTCLYECSPNLGPWIQQVDQSWRKERVLNVPLCKEDCEQWWEDCRTSYTCKSNWHKGWNWTSGFNKCAVGAACQPFHFYFPTPTVLCNEIWTHSYKVSNYSRGSGRCIQMWFDPAQGNPNEEVARFYAAAMSGAGPWAAWPFLLSLALMLLWLLS

SEQ ID NO: 16 - protein, 255 aa, artificial
  FRb with signal peptide
MVWKWMPLLLLLVCVATMCSAQDRTDLLNVCMDAKHHKTKPGPEDKLHDQCSPWKKNACCTASTSQELHKDTSRLYNFNWDHCGKMEPACKRHFIQDTCLYECSPNLGPWIQQVNQSWRKERFLDVPLCKEDCQRWWEDCHTSHTCKSNWHRGWDWTSGVNKCPAGALCRTFESYFPTPAALCEGLWSHSYKVSNYSRGSGRCIQMWFDSAQGNPNEEVARFYAAAMHVNAGEMLHGTGGLLLSLALMLQLWLLG

SEQ ID NO: 17 - protein, 335 aa, artificial
  uPAR with signal peptide
MGHPPLLPLLLLLHTCVPASWGLRCMQCKTNGDCRVEECALGQDLCRTTIVRLWEEGEELELVEKSCTHSEKTNRTLSYRTGLKITSLTEVVCGLDLCNQGNSGRAVTYSRSRYLECISCGSSDMSCERGRHQSLQCRSPEEQCLDVVTHWIQEGEEGRPKDDRHLRGCGYLPGCPGSNGFHNNDTFHFLKCCNTTKCNEGPILELENLPQNGRQCYSCKGNSTHGCSSEETFLIDCRGPMNQCLVATGTHEPKNQSYMVRGCATASMCQHAHLGDAFSMNHIDVSCCTKSGCNHPDLDVQYRSGAAPQPGPAHLSLTITLLMTARLWGGTLLWT

SEQ ID NO: 18 - protein, 187 aa, artificial
  DHFR
MVGSLNCIVAVSQNMGIGKNGDLPWPPLRNEFRYFQRMTTTSSVEGKQNLVIMGKKTWFSIPEKNRPLKGRINLVLSRELKEPPQGAHFLSRSLDDALKLTEQPELANKVDMVWIVGGSSVYKEAMNHPGHLKLFVTRIMQDFESDTFFPEIDLEKYKLLPEYPGVLSDVQEEKGIKYKFEVYEKND

SEQ ID NO: 19 - protein, 255 aa, artificial
  scFv against FITC: 4M5.3(Kd = 200pM)
DVVMTQTPLSLPVSLGDQASISCRSSQSLVHSNGNTYLRWYLQKPGQSPKVLIYKVSNRVSGVPDRFSGSGSGTDFTLKINRVEAEDLGVYFCSQSTHVPWTFGGGTKLEIKSSADDAKKDAAKKDDAKKDDAKKDGGVKLDETGGGLVQPGGAMKLSCVTSGFTFGHYWMNWVRQSPEKGLEWVAQFRNKPYNYETYYSDSVKGRFTISRDDSKSSVYLQMNNLRVEDTGIYYCTGASYGMEYLGQGTSVTVSS

SEQ ID NO: 20 - protein, 244 aa, artificial
  scFv against FITC 4D5Flu (Kd=10nM)
DIQMTQSPSSLSASVGDRVTITCRASQDVNTAVAWYQQKPGKAPKLLIYSASFLYSGVPSRFSGSRSGTDFTLTISSLQPEDFATYYCQQHYTTPPTFGQGTKVEIKRTGGGGSGGGGSGGGGSEVQLVESGGGLVQPGGSLRLSCAASGFNIKDTYIHWVRQAPGKGLEWVARIYPTNGYTRYADSVKGRFTISADTSKNTAYLQMNSLRAEDTAVYYCSRWGGDGFYAMDYWGQGTLVTVSS

SEQ ID NO: 21 - protein, 244 aa, artificial
  scFv against DNP SPE7
QAVVTQESALTTSPGETVTLTCRSSTGAVTTSNYANWVQEKPDHLFTGLIGGTNNRAPGVPARFSGSLIGDKAALTITGAQTEDEAIYFCALWYSNHLVFGGGTKLTVLGGGGSGGGGSGGGGSEVQLQQPGAELVKPGASVKLSCKASGYTFTSYWMHWVKQRPGRGLEWIGRIDPNGGGTKYNEKFKSKATLTVDKPSSTAYMQLSSLTSEDSAVYYCARMWYYGTYYFDYWGQGTTLTVSS